European Patent Specification EP 3 894 549 B1, published July 31, 2024. Title: Mutated piggyBac Transposases. Applicant: AMGEN INC. The sequence listing filed with the application follows.

SEQUENCE LISTING (18 sequences)

SEQ ID NO: 1 - DNA, 1786 bp, Trichoplusia ni
atgggctctagcctggacgacgagcacatcctgagcgccctgctgcagagcgacgacgaactggtgggcgaggacagcgacagcgagatcagcgaccacgtgtccgaggacgacgtgcagtccgacaccgaggaagccttcatcgacgaggtgcacgaagtgcagcctaccagcagcggctccgagatcctggacgagcagaacgtgatcgagcagcctggcagctccctggccagcaacagaatcctgaccctgccccagagaaccatcagaggcaagaacaagcactgctggtccacctccaagagcaccaggcggagcagagtgtccgccctgaacatcgtgcggagccagaggggccccaccagaatgtgcagaaacatctacgaccccctgctgtgcttcaagctgttcttcaccgacgagatcatcagcgagatcgtgaagtggaccaacgccgagatcagcctgaagaggcgggagagcatgaccggcgccaccttcagagacaccaacgaggacgagatctacgccttcttcggcatcctggtgatgaccgccgtgagaaaggacaaccacatgagcaccgacgacctgttcgacagatccctgagcatggtgtacgtgtccgtgatgagcagagacagattcgacttcctgatcagatgcctgagaatggacgacaagagcatcagacccaccctgcgggagaacgacgtgttcacccccgtgcggaagatctgggacctgttcatccaccagtgcatccagaactacacccctggcgcccacctgaccatcgatgagcagctgctgggcttcagaggcagatgccccttcagaatgtacatccccaacaagcccagcaagtacggcatcaagatcctgatgatgtgcgacagcggcaccaagtacatgatcaacggcatgccctacctgggcagaggcacccagacaaacggcgtgcccctgggcgagtactacgtgaaagaactgagcaagcctgtgcatggcagctgcaggaacatcacctgcgacaactggttcaccagcatccccctggccaagaacctgctgcaggaaccctacaagctgaccatcgtgggcaccgtgcggagcaacaagcgggagatcccagaggtgctgaagaacagcagatccagacctgtgggaacaagcatgttctgcttcgacggccccctgaccctggtgtcctacaagcccaagcccgccaagatggtgtacctgctgtccagctgcgacgaggacgccagcatcaacgagagcaccggcaagccccagatggtgatgtactacaaccagaccaagggcggcgtggacaccctggaccagatgtgcagcgtgatgacctgcagcagaaagaccaacagatggcccatggccctgctgtacggcatgatcaatatcgcctgcatcaacagcttcatcatctacagccacaacgtgtccagcaagggcgagaaggtgcagagccggaagaaattcatgcggaacctgtacatgagcctgacctccagcttcatgagaaagagactggaagcccccaccctgaagagatacctgcgggacaacatcagcaacatcctgcccaacgaagtgccaggaacaagcgacgacagcaccgaggaacccgtgatgaagaagaggacctactgcacctactgtcccagcaagatcagaagaaaggccaacgccagctgcaagaaatgcaaaaaagtgatctgccgggagcacaacatcgacatgtgccagagctgtttctagc

SEQ ID NO: 2 - protein, 594 aa, Trichoplusia ni
MGSSLDDEHILSALLQSDDELVGEDSDSEISDHVSEDDVQSDTEEAFIDEVHEVQPTSSGSEILDEQNVIEQPGSSLASNRILTLPQRTIRGKNKHCWSTSKSTRRSRVSALNIVRSQRGPTRMCRNIYDPLLCFKLFFTDEIISEIVKWTNAEISLKRRESMTGATFRDTNEDEIYAFFGILVMTAVRKDNHMSTDDLFDRSLSMVYVSVMSRDRFDFLIRCLRMDDKSIRPTLRENDVFTPVRKIWDLFIHQCIQNYTPGAHLTIDEQLLGFRGRCPFRMYIPNKPSKYGIKILMMCDSGTKYMINGMPYLGRGTQTNGVPLGEYYVKELSKPVHGSCRNITCDNWFTSIPLAKNLLQEPYKLTIVGTVRSNKREIPEVLKNSRSRPVGTSMFCFDGPLTLVSYKPKPAKMVYLLSSCDEDASINESTGKPQMVMYYNQTKGGVDTLDQMCSVMTCSRKTNRWPMALLYGMINIACINSFIIYSHNVSSKGEKVQSRKKFMRNLYMSLTSSFMRKRLEAPTLKRYLRDNISNILPNEVPGTSDDSTEEPVMKKRTYCTYCPSKIRRKANASCKKCKKVICREHNIDMCQSCF

SEQ ID NO: 3 - DNA, 1786 bp, Trichoplusia ni
atgggctctagcctggacgacgagcacatcctgagcgccctgctgcagagcgacgacgaactggtgggcgaggacagcgacagcgagatcagcgaccacgtgtccgaggacgacgtgcagtccgacaccgaggaagccttcatcgacgaggtgcacgaagtgcagcctaccagcagcggctccgagatcctggacgagcagaacgtgatcgagcagcctggcagctccctggccagcaacagaatcctgaccctgccccagagaaccatcagaggcaagaacaagcactgctggtccacctccaagagcaccaggcggagcagagtgtccgccctgaacatcgtgcggagccagaggggccccaccagaatgtgcagaaacatctacgaccccctgctgtgcttcaagctgttcttcaccgacgagatcatcagcgagctggtgaagtggaccaacgccgagatcagcctgaagaggcgggagagcatgaccggcgccaccttcagagacaccaacgaggacgagatctacgccttcttcggcatcctggtgatgaccgccgtgagaaaggacaaccacatgagcaccgacgacctgttcgacagatccctgagcatggtgtacgtgtccgtgatgagcagagacagattcgacttcctgatcagatgcctgagaatggacgacaagagcatcagacccaccctgcgggagaacgacgtgttcacccccgtgcggaagatctgggacctgttcatccaccagtgcatccagaactacacccctggcgcccacctgaccatcgatgagcagctgctgggcttcagaggcagatgccccttcagaatgtacatccccaacaagcccagcaagtacggcatcaagatcctgatgatgtgcgacagcggcaccaagtacatgatcaacggcatgccctacctgggcagaggcacccagacaaacggcgtgcccctgggcgagtactacgtgaaagaactgagcaagcctgtgcatggcagctgcaggaacatcacctgcgacaactggttcaccagcatccccctggccaagaacctgctgcaggaaccctacaagctgaccatcgtgggcaccgtgcggagcaacaagcgggagatcccagaggtgctgaagaacagcagatccagacctgtgggaacaagcatgttctgcttcgacggccccctgaccctggtgtcctacaagcccaagcccgccaagatggtgtacctgctgtccagctgcgacgaggacgccagcatcaacgagagcaccggcaagccccagatggtgatgtactacaaccagaccaagggcggcgtggacaccctggaccagatgtgcagcgtgatgacctgcagcagaaagaccaacagatggcccatggccctgctgtacggcatgatcaatatcgcctgcatcaacagcttcatcatctacagccacaacgtgtccagcaagggcgagaaggtgcagagccggaagaaattcatgcggaacctgtacatgagcctgacctccagcttcatgagaaagagactggaagcccccaccctgaagagatacctgcgggacaacatcagcaacatcctgcccaacgaagtgccaggaacaagcgacgacagcaccgaggaacccgtgatgaagaagaggacctactgcacctactgtcccagcaagatcagaagaaaggccaacgccagctgcaagaaatgcaaaaaagtgatctgccgggagcacaacatcgacatgtgccagagctgtttctagc

SEQ ID NO: 4 - protein, 594 aa, Trichoplusia ni
MGSSLDDEHILSALLQSDDELVGEDSDSEISDHVSEDDVQSDTEEAFIDEVHEVQPTSSGSEILDEQNVIEQPGSSLASNRILTLPQRTIRGKNKHCWSTSKSTRRSRVSALNIVRSQRGPTRMCRNIYDPLLCFKLFFTDEIISELVKWTNAEISLKRRESMTGATFRDTNEDEIYAFFGILVMTAVRKDNHMSTDDLFDRSLSMVYVSVMSRDRFDFLIRCLRMDDKSIRPTLRENDVFTPVRKIWDLFIHQCIQNYTPGAHLTIDEQLLGFRGRCPFRMYIPNKPSKYGIKILMMCDSGTKYMINGMPYLGRGTQTNGVPLGEYYVKELSKPVHGSCRNITCDNWFTSIPLAKNLLQEPYKLTIVGTVRSNKREIPEVLKNSRSRPVGTSMFCFDGPLTLVSYKPKPAKMVYLLSSCDEDASINESTGKPQMVMYYNQTKGGVDTLDQMCSVMTCSRKTNRWPMALLYGMINIACINSFIIYSHNVSSKGEKVQSRKKFMRNLYMSLTSSFMRKRLEAPTLKRYLRDNISNILPNEVPGTSDDSTEEPVMKKRTYCTYCPSKIRRKANASCKKCKKVICREHNIDMCQSCF

SEQ ID NO: 5 - DNA, 1786 bp, Trichoplusia ni
atgggctctagcctggacgacgagcacatcctgagcgccctgctgcagagcgacgacgaactggtgggcgaggacagcgacagcgagatcagcgaccacgtgtccgaggacgacgtgcagtccgacaccgaggaagccttcatcgacgaggtgcacgaagtgcagcctaccagcagcggctccgagatcctggacgagcagaacgtgatcgagcagcctggcagctccctggccagcaacagaatcctgaccctgccccagagaaccatcagaggcaagaacaagcactgctggtccacctccaagagcaccaggcggagcagagtgtccgccctgaacatcgtgcggagccagaggggccccaccagaatgtgcagaaacatctacgaccccctgctgtgcttcaagctgttcttcaccgacgagatcatcagcgagatcgtgaagtggaccaacgccgagatcagcctgaagaggcgggagagcatgaccggcgccaccttcagagacaccaacgaggacgagatctacgccttcttcggcatcctggtgatgaccgccgtgagaaaggacaaccacatgagcaccgacgacctgttcgacagatccctgagcatggtgtacgtgtccgtgatgagcagagacagattcgacttcctgatcagatgcctgagaatggacgacaagagcatcagacccaccctgcgggagaacgacgtgttcacccccgtgcggaagctgtgggacctgttcatccaccagtgcatccagaactacacccctggcgcccacctgaccatcgatgagcagctgctgggcttcagaggcagatgccccttcagaatgtacatccccaacaagcccagcaagtacggcatcaagatcctgatgatgtgcgacagcggcaccaagtacatgatcaacggcatgccctacctgggcagaggcacccagacaaacggcgtgcccctgggcgagtactacgtgaaagaactgagcaagcctgtgcatggcagctgcaggaacatcacctgcgacaactggttcaccagcatccccctggccaagaacctgctgcaggaaccctacaagctgaccatcgtgggcaccgtgcggagcaacaagcgggagatcccagaggtgctgaagaacagcagatccagacctgtgggaacaagcatgttctgcttcgacggccccctgaccctggtgtcctacaagcccaagcccgccaagatggtgtacctgctgtccagctgcgacgaggacgccagcatcaacgagagcaccggcaagccccagatggtgatgtactacaaccagaccaagggcggcgtggacaccctggaccagatgtgcagcgtgatgacctgcagcagaaagaccaacagatggcccatggccctgctgtacggcatgatcaatatcgcctgcatcaacagcttcatcatctacagccacaacgtgtccagcaagggcgagaaggtgcagagccggaagaaattcatgcggaacctgtacatgagcctgacctccagcttcatgagaaagagactggaagcccccaccctgaagagatacctgcgggacaacatcagcaacatcctgcccaacgaagtgccaggaacaagcgacgacagcaccgaggaacccgtgatgaagaagaggacctactgcacctactgtcccagcaagatcagaagaaaggccaacgccagctgcaagaaatgcaaaaaagtgatctgccgggagcacaacatcgacatgtgccagagctgtttctagc

SEQ ID NO: 6 - protein, 594 aa, Trichoplusia ni
MGSSLDDEHILSALLQSDDELVGEDSDSEISDHVSEDDVQSDTEEAFIDEVHEVQPTSSGSEILDEQNVIEQPGSSLASNRILTLPQRTIRGKNKHCWSTSKSTRRSRVSALNIVRSQRGPTRMCRNIYDPLLCFKLFFTDEIISEIVKWTNAEISLKRRESMTGATFRDTNEDEIYAFFGILVMTAVRKDNHMSTDDLFDRSLSMVYVSVMSRDRFDFLIRCLRMDDKSIRPTLRENDVFTPVRKLWDLFIHQCIQNYTPGAHLTIDEQLLGFRGRCPFRMYIPNKPSKYGIKILMMCDSGTKYMINGMPYLGRGTQTNGVPLGEYYVKELSKPVHGSCRNITCDNWFTSIPLAKNLLQEPYKLTIVGTVRSNKREIPEVLKNSRSRPVGTSMFCFDGPLTLVSYKPKPAKMVYLLSSCDEDASINESTGKPQMVMYYNQTKGGVDTLDQMCSVMTCSRKTNRWPMALLYGMINIACINSFIIYSHNVSSKGEKVQSRKKFMRNLYMSLTSSFMRKRLEAPTLKRYLRDNISNILPNEVPGTSDDSTEEPVMKKRTYCTYCPSKIRRKANASCKKCKKVICREHNIDMCQSCF

SEQ ID NO: 7 - DNA, 1786 bp, Trichoplusia ni
atgggctctagcctggacgacgagcacatcctgagcgccctgctgcagagcgacgacgaactggtgggcgaggacagcgacagcgagatcagcgaccacgtgtccgaggacgacgtgcagtccgacaccgaggaagccttcatcgacgaggtgcacgaagtgcagcctaccagcagcggctccgagatcctggacgagcagaacgtgatcgagcagcctggcagctccctggccagcaacagaatcctgaccctgccccagagaaccatcagaggcaagaacaagcactgctggtccacctccaagagcaccaggcggagcagagtgtccgccctgaacatcgtgcggagccagaggggccccaccagaatgtgcagaaacatctacgaccccctgctgtgcttcaagctgttcttcaccgacgagatcatcagcgagatcgtgaagtggaccaacgccgagatcagcctgaagaggcgggagagcatgaccggcgccaccttcagagacaccaacgaggacgagatctacgccttcttcggcatcctggtgatgaccgccgtgagaaaggacaaccacatgagcaccgacgacctgttcgacagatccctgagcatggtgtacgtgtccgtgatgagcagagacagattcgacttcctgatcagatgcctgagaatggacgacaagagcatcagacccaccctgcgggagaacgacgtgttcacccccgtgcggaagatctgggacctgttcatccaccagtgcatccagaactacacccctggcgcccacctgaccatcgatgagcagctgctgggcttcagaggcagatgccccttcagaatgtacatccccaacaagcccagcaagtacggcatcaagatcctgatgatgtgcgacagcggcaccaagtacatgatcaacggcatgccctacctgggcagaggcacccagacaaacggcgtgcccctgggcgagtactacgtgaaagaactgagcaagcctgtgcatggcagctgcaggaacatcacctgcgacaactggttcaccagcatccccctggccaagaacctgctgcaggaaccctacaagctgaccatcgtgggcaccgtgcggagcaacaagcgggagatcccagaggtgctgaagaacagcagatccagacctgtgggaacaagcatgttctgcttcgacggccccctgaccctggtgtcctacaagcccaagcccgccaagatggtgtacctgctgtccagctgcgacgaggacgccagcatcaacgagagcaccggcaagccccagatggtgatgtactacaaccagaccaagggcggcgtggacaccctggaccagatgtgcagcgtgatgacctgcagcagaaagaccaacagatggcccatggccctgctgtacggcatgatcaatatcgcctgcatcaacagcttcatcatctacagccacaacgtgtccagcaagggcgagaaggtgcagagccggaagaaattcatgcggaacctgtacatgagcctgacctccagcttcatgagaaagagactggaagcccccaccctgaagagatacctgcgggacaacatcaccaacatcctgcccaacgaagtgccaggaacaagcgacgacagcaccgaggaacccgtgatgaagaagaggacctactgcacctactgtcccagcaagatcagaagaaaggccaacgccagctgcaagaaatgcaaaaaagtgatctgccgggagcacaacatcgacatgtgccagagctgtttctagc

SEQ ID NO: 8 - protein, 594 aa, Trichoplusia ni
MGSSLDDEHILSALLQSDDELVGEDSDSEISDHVSEDDVQSDTEEAFIDEVHEVQPTSSGSEILDEQNVIEQPGSSLASNRILTLPQRTIRGKNKHCWSTSKSTRRSRVSALNIVRSQRGPTRMCRNIYDPLLCFKLFFTDEIISEIVKWTNAEISLKRRESMTGATFRDTNEDEIYAFFGILVMTAVRKDNHMSTDDLFDRSLSMVYVSVMSRDRFDFLIRCLRMDDKSIRPTLRENDVFTPVRKIWDLFIHQCIQNYTPGAHLTIDEQLLGFRGRCPFRMYIPNKPSKYGIKILMMCDSGTKYMINGMPYLGRGTQTNGVPLGEYYVKELSKPVHGSCRNITCDNWFTSIPLAKNLLQEPYKLTIVGTVRSNKREIPEVLKNSRSRPVGTSMFCFDGPLTLVSYKPKPAKMVYLLSSCDEDASINESTGKPQMVMYYNQTKGGVDTLDQMCSVMTCSRKTNRWPMALLYGMINIACINSFIIYSHNVSSKGEKVQSRKKFMRNLYMSLTSSFMRKRLEAPTLKRYLRDNITNILPNEVPGTSDDSTEEPVMKKRTYCTYCPSKIRRKANASCKKCKKVICREHNIDMCQSCF

SEQ ID NO: 9 - DNA, 1786 bp, Trichoplusia ni
atgggctctagcctggacgacgagcacatcctgagcgccctgctgcagagcgacgacgaactggtgggcgaggacagcgacagcgagatcagcgaccacgtgtccgaggacgacgtgcagtccgacaccgaggaagccttcatcgacgaggtgcacgaagtgcagcctaccagcagcggctccgagatcctggacgagcagaacgtgatcgagcagcctggcagctccctggccagcaacagaatcctgaccctgccccagagaaccatcagaggcaagaacaagcactgctggtccacctccaagagcaccaggcggagcagagtgtccgccctgaacatcgtgcggagccagaggggccccaccagaatgtgcagaaacatctacgaccccctgctgtgcttcaagctgttcttcaccgacgagatcatcagcgagctggtgaagtggaccaacgccgagatcagcctgaagaggcgggagagcatgaccggcgccaccttcagagacaccaacgaggacgagatctacgccttcttcggcatcctggtgatgaccgccgtgagaaaggacaaccacatgagcaccgacgacctgttcgacagatccctgagcatggtgtacgtgtccgtgatgagcagagacagattcgacttcctgatcagatgcctgagaatggacgacaagagcatcagacccaccctgcgggagaacgacgtgttcacccccgtgcggaagctgtgggacctgttcatccaccagtgcatccagaactacacccctggcgcccacctgaccatcgatgagcagctgctgggcttcagaggcagatgccccttcagaatgtacatccccaacaagcccagcaagtacggcatcaagatcctgatgatgtgcgacagcggcaccaagtacatgatcaacggcatgccctacctgggcagaggcacccagacaaacggcgtgcccctgggcgagtactacgtgaaagaactgagcaagcctgtgcatggcagctgcaggaacatcacctgcgacaactggttcaccagcatccccctggccaagaacctgctgcaggaaccctacaagctgaccatcgtgggcaccgtgcggagcaacaagcgggagatcccagaggtgctgaagaacagcagatccagacctgtgggaacaagcatgttctgcttcgacggccccctgaccctggtgtcctacaagcccaagcccgccaagatggtgtacctgctgtccagctgcgacgaggacgccagcatcaacgagagcaccggcaagccccagatggtgatgtactacaaccagaccaagggcggcgtggacaccctggaccagatgtgcagcgtgatgacctgcagcagaaagaccaacagatggcccatggccctgctgtacggcatgatcaatatcgcctgcatcaacagcttcatcatctacagccacaacgtgtccagcaagggcgagaaggtgcagagccggaagaaattcatgcggaacctgtacatgagcctgacctccagcttcatgagaaagagactggaagcccccaccctgaagagatacctgcgggacaacatcaccaacatcctgcccaacgaagtgccaggaacaagcgacgacagcaccgaggaacccgtgatgaagaagaggacctactgcacctactgtcccagcaagatcagaagaaaggccaacgccagctgcaagaaatgcaaaaaagtgatctgccgggagcacaacatcgacatgtgccagagctgtttctagc

SEQ ID NO: 10 - protein, 594 aa, Trichoplusia ni
MGSSLDDEHILSALLQSDDELVGEDSDSEISDHVSEDDVQSDTEEAFIDEVHEVQPTSSGSEILDEQNVIEQPGSSLASNRILTLPQRTIRGKNKHCWSTSKSTRRSRVSALNIVRSQRGPTRMCRNIYDPLLCFKLFFTDEIISELVKWTNAEISLKRRESMTGATFRDTNEDEIYAFFGILVMTAVRKDNHMSTDDLFDRSLSMVYVSVMSRDRFDFLIRCLRMDDKSIRPTLRENDVFTPVRKLWDLFIHQCIQNYTPGAHLTIDEQLLGFRGRCPFRMYIPNKPSKYGIKILMMCDSGTKYMINGMPYLGRGTQTNGVPLGEYYVKELSKPVHGSCRNITCDNWFTSIPLAKNLLQEPYKLTIVGTVRSNKREIPEVLKNSRSRPVGTSMFCFDGPLTLVSYKPKPAKMVYLLSSCDEDASINESTGKPQMVMYYNQTKGGVDTLDQMCSVMTCSRKTNRWPMALLYGMINIACINSFIIYSHNVSSKGEKVQSRKKFMRNLYMSLTSSFMRKRLEAPTLKRYLRDNITNILPNEVPGTSDDSTEEPVMKKRTYCTYCPSKIRRKANASCKKCKKVICREHNIDMCQSCF

SEQ ID NO: 11 - DNA, 1786 bp, Trichoplusia ni
atgggctctagcctggacgacgagcacatcctgagcgccctgctgcagagcgacgacgaactggtgggcgaggacagcgacagcgagatcagcgaccacgtgtccgaggacgacgtgcagtccgacaccgaggaagccttcatcgacgaggtgcacgaagtgcagcctaccagcagcggctccgagatcctggacgagcagaacgtgatcgagcagcctggcagctccctggccagcaacagaatcctgaccctgccccagagaaccatcagaggcaagaacaagcactgctggtccacctccaagagcaccaggcggagcagagtgtccgccctgaacatcgtgcggagccagaggggccccaccagaatgtgcagaaacatctacgaccccctgctgtgcttcaagctgttcttcaccgacgagatcatcagcgagatcgtgaagtggaccaacgccgagatcagcctgaagaggcgggagagcatgaccggcgccaccttcagagacaccaacgaggacgagatctacgccttcttcggcatcctggtgatgaccgccgtgagaaaggacaaccacatgagcaccgacgacctgttcgacagatccctgagcatggtgtacgtgtccgtgatgagcagagacagattcgacttcctgatcagatgcctgagaatggacgacaagagcatcagacccaccctgcgggagaacgacgtgttcacccccgtgcggaagctgtgggacctgttcatccaccagtgcatccagaactacacccctggcgcccacctgaccatcgatgagcagctgctgggcttcagaggcagatgccccttcagaatgtacatccccaacaagcccagcaagtacggcatcaagatcctgatgatgtgcgacagcggcaccaagtacatgatcaacggcatgccctacctgggcagaggcacccagacaaacggcgtgcccctgggcgagtactacgtgaaagaactgagcaagcctgtgcatggcagctgcaggaacatcacctgcgacaactggttcaccagcatccccctggccaagaacctgctgcaggaaccctacaagctgaccatcgtgggcaccgtgcggagcaacaagcgggagatcccagaggtgctgaagaacagcagatccagacctgtgggaacaagcatgttctgcttcgacggccccctgaccctggtgtcctacaagcccaagcccgccaagatggtgtacctgctgtccagctgcgacgaggacgccagcatcaacgagagcaccggcaagccccagatggtgatgtactacaaccagaccaagggcggcgtggacaccctggaccagatgtgcagcgtgatgacctgcagcagaaagaccaacagatggcccatggccctgctgtacggcatgatcaatatcgcctgcatcaacagcttcatcatctacagccacaacgtgtccagcaagggcgagaaggtgcagagccggaagaaattcatgcggaacctgtacatgagcctgacctccagcttcatgagaaagagactggaagcccccaccctgaagagatacctgcgggacaacatcaccaacatcctgcccaacgaagtgccaggaacaagcgacgacagcaccgaggaacccgtgatgaagaagaggacctactgcacctactgtcccagcaagatcagaagaaaggccaacgccagctgcaagaaatgcaaaaaagtgatctgccgggagcacaacatcgacatgtgccagagctgtttctagc

SEQ ID NO: 12 - protein, 594 aa, Trichoplusia ni
MGSSLDDEHILSALLQSDDELVGEDSDSEISDHVSEDDVQSDTEEAFIDEVHEVQPTSSGSEILDEQNVIEQPGSSLASNRILTLPQRTIRGKNKHCWSTSKSTRRSRVSALNIVRSQRGPTRMCRNIYDPLLCFKLFFTDEIISEIVKWTNAEISLKRRESMTGATFRDTNEDEIYAFFGILVMTAVRKDNHMSTDDLFDRSLSMVYVSVMSRDRFDFLIRCLRMDDKSIRPTLRENDVFTPVRKLWDLFIHQCIQNYTPGAHLTIDEQLLGFRGRCPFRMYIPNKPSKYGIKILMMCDSGTKYMINGMPYLGRGTQTNGVPLGEYYVKELSKPVHGSCRNITCDNWFTSIPLAKNLLQEPYKLTIVGTVRSNKREIPEVLKNSRSRPVGTSMFCFDGPLTLVSYKPKPAKMVYLLSSCDEDASINESTGKPQMVMYYNQTKGGVDTLDQMCSVMTCSRKTNRWPMALLYGMINIACINSFIIYSHNVSSKGEKVQSRKKFMRNLYMSLTSSFMRKRLEAPTLKRYLRDNITNILPNEVPGTSDDSTEEPVMKKRTYCTYCPSKIRRKANASCKKCKKVICREHNIDMCQSCF

SEQ ID NO: 13 - DNA, 1786 bp, Trichoplusia ni
atgggctctagcctggacgacgagcacatcctgagcgccctgctgcagagcgacgacgaactggtgggcgaggacagcgacagcgagatcagcgaccacgtgtccgaggacgacgtgcagtccgacaccgaggaagccttcatcgacgaggtgcacgaagtgcagcctaccagcagcggctccgagatcctggacgagcagaacgtgatcgagcagcctggcagctccctggccagcaacagaatcctgaccctgccccagagaaccatcagaggcaagaacaagcactgctggtccacctccaagagcaccaggcggagcagagtgtccgccctgaacatcgtgcggagccagaggggccccaccagaatgtgcagaaacatctacgaccccctgctgtgcttcaagctgttcttcaccgacgagatcatcagcgagctggtgaagtggaccaacgccgagatcagcctgaagaggcgggagagcatgaccggcgccaccttcagagacaccaacgaggacgagatctacgccttcttcggcatcctggtgatgaccgccgtgagaaaggacaaccacatgagcaccgacgacctgttcgacagatccctgagcatggtgtacgtgtccgtgatgagcagagacagattcgacttcctgatcagatgcctgagaatggacgacaagagcatcagacccaccctgcgggagaacgacgtgttcacccccgtgcggaagatctgggacctgttcatccaccagtgcatccagaactacacccctggcgcccacctgaccatcgatgagcagctgctgggcttcagaggcagatgccccttcagaatgtacatccccaacaagcccagcaagtacggcatcaagatcctgatgatgtgcgacagcggcaccaagtacatgatcaacggcatgccctacctgggcagaggcacccagacaaacggcgtgcccctgggcgagtactacgtgaaagaactgagcaagcctgtgcatggcagctgcaggaacatcacctgcgacaactggttcaccagcatccccctggccaagaacctgctgcaggaaccctacaagctgaccatcgtgggcaccgtgcggagcaacaagcgggagatcccagaggtgctgaagaacagcagatccagacctgtgggaacaagcatgttctgcttcgacggccccctgaccctggtgtcctacaagcccaagcccgccaagatggtgtacctgctgtccagctgcgacgaggacgccagcatcaacgagagcaccggcaagccccagatggtgatgtactacaaccagaccaagggcggcgtggacaccctggaccagatgtgcagcgtgatgacctgcagcagaaagaccaacagatggcccatggccctgctgtacggcatgatcaatatcgcctgcatcaacagcttcatcatctacagccacaacgtgtccagcaagggcgagaaggtgcagagccggaagaaattcatgcggaacctgtacatgagcctgacctccagcttcatgagaaagagactggaagcccccaccctgaagagatacctgcgggacaacatcaccaacatcctgcccaacgaagtgccaggaacaagcgacgacagcaccgaggaacccgtgatgaagaagaggacctactgcacctactgtcccagcaagatcagaagaaaggccaacgccagctgcaagaaatgcaaaaaagtgatctgccgggagcacaacatcgacatgtgccagagctgtttctagc

SEQ ID NO: 14 - protein, 594 aa, Trichoplusia ni
MGSSLDDEHILSALLQSDDELVGEDSDSEISDHVSEDDVQSDTEEAFIDEVHEVQPTSSGSEILDEQNVIEQPGSSLASNRILTLPQRTIRGKNKHCWSTSKSTRRSRVSALNIVRSQRGPTRMCRNIYDPLLCFKLFFTDEIISELVKWTNAEISLKRRESMTGATFRDTNEDEIYAFFGILVMTAVRKDNHMSTDDLFDRSLSMVYVSVMSRDRFDFLIRCLRMDDKSIRPTLRENDVFTPVRKIWDLFIHQCIQNYTPGAHLTIDEQLLGFRGRCPFRMYIPNKPSKYGIKILMMCDSGTKYMINGMPYLGRGTQTNGVPLGEYYVKELSKPVHGSCRNITCDNWFTSIPLAKNLLQEPYKLTIVGTVRSNKREIPEVLKNSRSRPVGTSMFCFDGPLTLVSYKPKPAKMVYLLSSCDEDASINESTGKPQMVMYYNQTKGGVDTLDQMCSVMTCSRKTNRWPMALLYGMINIACINSFIIYSHNVSSKGEKVQSRKKFMRNLYMSLTSSFMRKRLEAPTLKRYLRDNITNILPNEVPGTSDDSTEEPVMKKRTYCTYCPSKIRRKANASCKKCKKVICREHNIDMCQSCF

SEQ ID NO: 15 - DNA, 1786 bp, Trichoplusia ni
atgggctctagcctggacgacgagcacatcctgagcgccctgctgcagagcgacgacgaactggtgggcgaggacagcgacagcgagatcagcgaccacgtgtccgaggacgacgtgcagtccgacaccgaggaagccttcatcgacgaggtgcacgaagtgcagcctaccagcagcggctccgagatcctggacgagcagaacgtgatcgagcagcctggcagctccctggccagcaacagaatcctgaccctgccccagagaaccatcagaggcaagaacaagcactgctggtccacctccaagagcaccaggcggagcagagtgtccgccctgaacatcgtgcggagccagaggggccccaccagaatgtgcagaaacatctacgaccccctgctgtgcttcaagctgttcttcaccgacgagatcatcagcgagctggtgaagtggaccaacgccgagatcagcctgaagaggcgggagagcatgaccggcgccaccttcagagacaccaacgaggacgagatctacgccttcttcggcatcctggtgatgaccgccgtgagaaaggacaaccacatgagcaccgacgacctgttcgacagatccctgagcatggtgtacgtgtccgtgatgagcagagacagattcgacttcctgatcagatgcctgagaatggacgacaagagcatcagacccaccctgcgggagaacgacgtgttcacccccgtgcggaagctgtgggacctgttcatccaccagtgcatccagaactacacccctggcgcccacctgaccatcgatgagcagctgctgggcttcagaggcagatgccccttcagaatgtacatccccaacaagcccagcaagtacggcatcaagatcctgatgatgtgcgacagcggcaccaagtacatgatcaacggcatgccctacctgggcagaggcacccagacaaacggcgtgcccctgggcgagtactacgtgaaagaactgagcaagcctgtgcatggcagctgcaggaacatcacctgcgacaactggttcaccagcatccccctggccaagaacctgctgcaggaaccctacaagctgaccatcgtgggcaccgtgcggagcaacaagcgggagatcccagaggtgctgaagaacagcagatccagacctgtgggaacaagcatgttctgcttcgacggccccctgaccctggtgtcctacaagcccaagcccgccaagatggtgtacctgctgtccagctgcgacgaggacgccagcatcaacgagagcaccggcaagccccagatggtgatgtactacaaccagaccaagggcggcgtggacaccctggaccagatgtgcagcgtgatgacctgcagcagaaagaccaacagatggcccatggccctgctgtacggcatgatcaatatcgcctgcatcaacagcttcatcatctacagccacaacgtgtccagcaagggcgagaaggtgcagagccggaagaaattcatgcggaacctgtacatgagcctgacctccagcttcatgagaaagagactggaagcccccaccctgaagagatacctgcgggacaacatcagcaacatcctgcccaacgaagtgccaggaacaagcgacgacagcaccgaggaacccgtgatgaagaagaggacctactgcacctactgtcccagcaagatcagaagaaaggccaacgccagctgcaagaaatgcaaaaaagtgatctgccgggagcacaacatcgacatgtgccagagctgtttctagc

SEQ ID NO: 16 - protein, 594 aa, Trichoplusia ni
MGSSLDDEHILSALLQSDDELVGEDSDSEISDHVSEDDVQSDTEEAFIDEVHEVQPTSSGSEILDEQNVIEQPGSSLASNRILTLPQRTIRGKNKHCWSTSKSTRRSRVSALNIVRSQRGPTRMCRNIYDPLLCFKLFFTDEIISELVKWTNAEISLKRRESMTGATFRDTNEDEIYAFFGILVMTAVRKDNHMSTDDLFDRSLSMVYVSVMSRDRFDFLIRCLRMDDKSIRPTLRENDVFTPVRKLWDLFIHQCIQNYTPGAHLTIDEQLLGFRGRCPFRMYIPNKPSKYGIKILMMCDSGTKYMINGMPYLGRGTQTNGVPLGEYYVKELSKPVHGSCRNITCDNWFTSIPLAKNLLQEPYKLTIVGTVRSNKREIPEVLKNSRSRPVGTSMFCFDGPLTLVSYKPKPAKMVYLLSSCDEDASINESTGKPQMVMYYNQTKGGVDTLDQMCSVMTCSRKTNRWPMALLYGMINIACINSFIIYSHNVSSKGEKVQSRKKFMRNLYMSLTSSFMRKRLEAPTLKRYLRDNISNILPNEVPGTSDDSTEEPVMKKRTYCTYCPSKIRRKANASCKKCKKVICREHNIDMCQSCF

SEQ ID NO: 17 - RNA, 1786 nt, Trichoplusia ni
augggcucuagccuggacgacgagcacauccugagcgcccugcugcagagcgacgacgaacuggugggcgaggacagcgacagcgagaucagcgaccacguguccgaggacgacgugcaguccgacaccgaggaagccuucaucgacgaggugcacgaagugcagccuaccagcagcggcuccgagauccuggacgagcagaacgugaucgagcagccuggcagcucccuggccagcaacagaauccugacccugccccagagaaccaucagaggcaagaacaagcacugcugguccaccuccaagagcaccaggcggagcagaguguccgcccugaacaucgugcggagccagaggggccccaccagaaugugcagaaacaucuacgacccccugcugugcuucaagcuguucuucaccgacgagaucaucagcgagaucgugaaguggaccaacgccgagaucagccugaagaggcgggagagcaugaccggcgccaccuucagagacaccaacgaggacgagaucuacgccuucuucggcauccuggugaugaccgccgugagaaaggacaaccacaugagcaccgacgaccuguucgacagaucccugagcaugguguacguguccgugaugagcagagacagauucgacuuccugaucagaugccugagaauggacgacaagagcaucagacccacccugcgggagaacgacguguucacccccgugcggaagcugugggaccuguucauccaccagugcauccagaacuacaccccuggcgcccaccugaccaucgaugagcagcugcugggcuucagaggcagaugccccuucagaauguacauccccaacaagcccagcaaguacggcaucaagauccugaugaugugcgacagcggcaccaaguacaugaucaacggcaugcccuaccugggcagaggcacccagacaaacggcgugccccugggcgaguacuacgugaaagaacugagcaagccugugcauggcagcugcaggaacaucaccugcgacaacugguucaccagcaucccccuggccaagaaccugcugcaggaacccuacaagcugaccaucgugggcaccgugcggagcaacaagcgggagaucccagaggugcugaagaacagcagauccagaccugugggaacaagcauguucugcuucgacggcccccugacccugguguccuacaagcccaagcccgccaagaugguguaccugcuguccagcugcgacgaggacgccagcaucaacgagagcaccggcaagccccagauggugauguacuacaaccagaccaagggcggcguggacacccuggaccagaugugcagcgugaugaccugcagcagaaagaccaacagauggcccauggcccugcuguacggcaugaucaauaucgccugcaucaacagcuucaucaucuacagccacaacguguccagcaagggcgagaaggugcagagccggaagaaauucaugcggaaccuguacaugagccugaccuccagcuucaugagaaagagacuggaagcccccacccugaagagauaccugcgggacaacaucaccaacauccugcccaacgaagugccaggaacaagcgacgacagcaccgaggaacccgugaugaagaagaggaccuacugcaccuacugucccagcaagaucagaagaaaggccaacgccagcugcaagaaaugcaaaaaagugaucugccgggagcacaacaucgacaugugccagagcuguuucuagc

SEQ ID NO: 18 - RNA, 1786 nt, Trichoplusia ni
augggcucuagccuggacgacgagcacauccugagcgcccugcugcagagcgacgacgaacuggugggcgaggacagcgacagcgagaucagcgaccacguguccgaggacgacgugcaguccgacaccgaggaagccuucaucgacgaggugcacgaagugcagccuaccagcagcggcuccgagauccuggacgagcagaacgugaucgagcagccuggcagcucccuggccagcaacagaauccugacccugccccagagaaccaucagaggcaagaacaagcacugcugguccaccuccaagagcaccaggcggagcagaguguccgcccugaacaucgugcggagccagaggggccccaccagaaugugcagaaacaucuacgacccccugcugugcuucaagcuguucuucaccgacgagaucaucagcgagcuggugaaguggaccaacgccgagaucagccugaagaggcgggagagcaugaccggcgccaccuucagagacaccaacgaggacgagaucuacgccuucuucggcauccuggugaugaccgccgugagaaaggacaaccacaugagcaccgacgaccuguucgacagaucccugagcaugguguacguguccgugaugagcagagacagauucgacuuccugaucagaugccugagaauggacgacaagagcaucagacccacccugcgggagaacgacguguucacccccgugcggaagcugugggaccuguucauccaccagugcauccagaacuacaccccuggcgcccaccugaccaucgaugagcagcugcugggcuucagaggcagaugccccuucagaauguacauccccaacaagcccagcaaguacggcaucaagauccugaugaugugcgacagcggcaccaaguacaugaucaacggcaugcccuaccugggcagaggcacccagacaaacggcgugccccugggcgaguacuacgugaaagaacugagcaagccugugcauggcagcugcaggaacaucaccugcgacaacugguucaccagcaucccccuggccaagaaccugcugcaggaacccuacaagcugaccaucgugggcaccgugcggagcaacaagcgggagaucccagaggugcugaagaacagcagauccagaccugugggaacaagcauguucugcuucgacggcccccugacccugguguccuacaagcccaagcccgccaagaugguguaccugcuguccagcugcgacgaggacgccagcaucaacgagagcaccggcaagccccagauggugauguacuacaaccagaccaagggcggcguggacacccuggaccagaugugcagcgugaugaccugcagcagaaagaccaacagauggcccauggcccugcuguacggcaugaucaauaucgccugcaucaacagcuucaucaucuacagccacaacguguccagcaagggcgagaaggugcagagccggaagaaauucaugcggaaccuguacaugagccugaccuccagcuucaugagaaagagacuggaagcccccacccugaagagauaccugcgggacaacaucaccaacauccugcccaacgaagugccaggaacaagcgacgacagcaccgaggaacccgugaugaagaagaggaccuacugcaccuacugucccagcaagaucagaagaaaggccaacgccagcugcaagaaaugcaaaaaagugaucugccgggagcacaacaucgacaugugccagagcuguuucuagc